European Patent Specification EP 4 053 274 B1, published April 15, 2026. Title: Fructose 6-phosphate 3-epimerase and use of the same. Applicant: SYMYANG COOPERATION. The sequence listing filed with the application follows.

SEQUENCE LISTING (10 sequences)

SEQ ID NO: 1 - protein, 227 aa, Artificial Sequence
  Fructose 6-phosphate 3-epimerase
MKYGFAPSLMCMNILKLEEQIKILNKKADFYHVDIMDGHYVKNITLSPFFIQQIRPLATIPIDAHLMVENPNDFLDELKKAGTDYVSLHVETINKDVFRITNKIKSLGMKVGVVLNPATPIDEIKHYINRLDKITVMTVDPGFAGQAFIPEMLDKIRELKEIKEKEGYKYIIEIDGSCNEKTFAQLKEAGAEVFVVGSSGLFNKDEDLEKAWEMMMSDFNYSLSYKE

SEQ ID NO: 2 - DNA, 684 bp, Artificial Sequence
  Polynucleotide sequence for fructose 6-phosphate 3-epimerase
atgaaatacggcttcgcaccgtccctgatgtgcatgaacatcctgaaactggaagaacaaatcaaaattctgaacaaaaaagcggatttctaccacgtagacattatggatgggcactatgttaaaaacatcacgctgtctccgttctttatccaacagatccgcccgctggcgaccattccaatcgacgcgcatctgatggtcgagaacccgaacgactttctggacgaactgaaaaaagctggtactgactacgtgtctctgcacgtagaaaccattaacaaagatgttttccgcatcacgaacaaaatcaaatcgttaggtatgaaagttggcgtggttctgaaccctgcgactccgatcgacgaaatcaaacattacatcaaccgtctggacaaaatcactgttatgactgttgaccctggtttcgctggccaagcgttcatcccggaaatgctggacaaaatccgtgaactcaaggaaatcaaagaaaaagagggttacaaatacattattgaaatcgatggcagctgcaacgaaaagactttcgcccaactgaaagaagcgggtgcggaagttttcgtagtcggctctagcggcctgtttaacaaagatgaagacctggaaaaagcctgggaaatgatgatgtccgacttcaattacagcctgagctacaaagaatag

SEQ ID NO: 3 - DNA, 27 bp, Artificial Sequence
  Primer pET21_ClRP3E_F
tatacatatgaaatacggcttcgcacc

SEQ ID NO: 4 - DNA, 31 bp, Artificial Sequence
  Primer pET21_ClRP3E_R
ggtgctcgagttctttgtagctcaggctgta

SEQ ID NO: 5 - protein, 225 aa, Artificial Sequence
  Ribulose-phosphate 3-epimerase (RuFP3E)
MKVEFSPSLMCMDFLKMEEQFNILNDKVDMYHIDIMDGHFCKNITLSPDLVKTFSKVAKKPMDVHLMTTNPTDWIEKVAAAGAEYISPHAETINGDAFRVMNMIKSLGCKTGVVLNPATPLSYVKHYLNRIDLLTIMTVDVGFAGQPFIEEMLDKIKEAKELKEKYGYTYKIQIDGSCNPKTYKRMYDAGAEVLIVGSSGLFGLNEDLNKACDQMFEDFNRAIAE

SEQ ID NO: 6 - DNA, 678 bp, Artificial Sequence
  Polynucleotide seqence for ribulose-phosphate 3-epimerase (RuFP3E)
atgaaagtagaattttctccgtccctgatgtgcatggacttcctgaagatggaagaacagttcaacattctgaatgacaaagtggacatgtatcatatcgacatcatggacggccatttctgcaagaacatcaccctgtccccggatctggttaaaaccttttctaaggtagcgaaaaaaccgatggatgtgcacttgatgaccaccaacccgaccgattggatcgaaaaagttgccgcggcgggcgctgagtacattagtccgcacgccgaaaccattaatggtgatgctttccgcgtgatgaacatgatcaagagcctgggctgcaaaaccggcgtagtactgaacccggccaccccgctgtcctatgttaaacactatctgaaccgcattgacctgctgaccattatgactgtagacgttggtttcgcgggccagccgttcatcgaggaaatgctggataaaatcaaagaagctaaagaactgaaagagaaatatggttacacctacaagatccagatcgacggctcttgcaacccgaaaacctataagcgtatgtacgacgcaggcgctgaagttctgattgtgggttctagcggtctgttcggtctgaacgaagatctgaacaaggcatgtgatcagatgttcgaagacttcaaccgtgcgatcgcagaataa

SEQ ID NO: 7 - protein, 225 aa, Artificial Sequence
  Ribulose-phosphate 3-epimerase (CDFP3E)
MKPMFAPSLMCANFLDLKNQIEILNERADIFHVDIMDGHYVKNFSLSPAMMEQLKTITKIPMDAHLMVENPADFLEGIAKAGATYISPHAETINKDAFRIMRTIKALGCKTGVVLNPATPVEYIKHYLGMLDKITILTVDAGFAGQTFIEEMLDKIEEVKRLREENGYSYLIEVDGSCNEKTFKKLAEAGTEVFIVGSSGLFNLDADLKVSWDKMMNMFNKCINN

SEQ ID NO: 8 - DNA, 678 bp, Artificial Sequence
  Polynucleotide sequence for ribulose-phosphate 3-epimerase (CDFP3E)
atgaagccgatgtttgctccgtctctgatgtgcgctaactttctcgatctcaaaaaccaaatcgaaatcttgaacgaacgcgctgacatcttccatgtagacatcatggatggccattacgtaaagaatttttctctctctccggcgatgatggaacagcttaaaaccattactaaaatcccgatggacgcccacctgatggtggaaaacccggcggatttcctggaaggaatcgcaaaagcgggcgcgacctacatcagccctcacgccgaaaccattaacaaagatgcgtttcgtatcatgcgcaccatcaaagctctgggctgtaaaactggtgttgtgctgaatccggccactccggtagagtacattaaacactatctgggcatgctggacaaaattaccatcctgactgttgacgcaggtttcgcgggtcagacctttatcgaagagatgctggataaaattgaagaagttaaacgtctgcgtgaagaaaacggttactcgtatttaattgaggtcgacggttcctgcaacgagaagactttcaaaaaattagcggaagctggtaccgaagttttcattgttggctctagcggcctgttcaacctggacgcggacctgaaagtgagctgggataaaatgatgaacatgttcaataaatgtatcaacaactaa

SEQ ID NO: 9 - protein, 228 aa, Artificial Sequence
  Ribulose-phosphate 3-epimerase (PkFP3E)
MKKHLFSPSLMCMNLMDIENQLKVLNQRADMVHIDIMDGHYVKNITLSPYFMEQIRESLTIPMDVHLMVEKPSEFIKMIIDAGATYISPHAEVINSEAFRMIDTIKSAGCKAGIALNPATPLSHIQHYIHHLDKITFMSVDPGFAGQKFIPEVLDKIREARALKEKHGYNYLIEIDGSCNEKTFKILEEAGVEVFIVGTSGLFNLDSDLNKAWDQMMEHFNSQVNAEV

SEQ ID NO: 10 - DNA, 687 bp, Artificial Sequence
  Polynucleotide sequence for ribulose-phosphate 3-epimerase (PkFP3E)
atgaaaaaacacctgttcagcccgtctctgatgtgtatgaatctgatggacatcgaaaaccagctgaaagtactgaatcagcgcgcagacatggtacacattgatatcatggatggccattatgttaaaaacattaccctgagcccgtacttcatggaacagattcgcgaatcgctgactatccctatggatgttcatctgatggttgaaaaaccgagcgaattcattaaaatgattatcgatgcgggtgccacctacattagccctcatgctgaagttatcaactctgaagcgtttcgtatgatcgacaccatcaaatccgcgggttgcaaagctggtattgcactgaacccggcaaccccgctgtctcacatccaacattacatccatcatctcgacaagatcacctttatgtccgttgatcctggtttcgctgggcagaaattcatccctgaagtcctggataagattcgtgaagctcgtgcactgaaagaaaaacacggctacaactacttaatcgaaatcgatggttcttgcaatgagaaaacctttaagatcctcgaagaagcaggtgtagaagttttcatcgttggtacttcgggactgttcaacctggatagcgacctgaacaaggcttgggaccagatgatggaacatttcaactctcaggtcaacgcagaggtctga